European Patent Specification EP 4 247 408 B1, published December 18, 2024. Title: Inhibitors of the Tissue Factor-Protease Activated Receptor 2 (TF-PAR2) signaling pathway for use in the treatment or prevention of heart failure (HF) and associated or resulting diseases. Applicant: Universitätsmedizin der Johannes Gutenberg-Universität Mainz. The sequence listing filed with the application follows.

SEQUENCE LISTING (2 sequences)

SEQ ID NO: 1 - protein, 84 aa, Ancylostoma caninum
KATMQCGENEKYDSCGSKECDKKCKYDGVEEEDDEEPNVPCLVRVCHQDCVCEEGFYRNKDDKCVSAEDCELDNMDFIYPGTRN

SEQ ID NO: 2 - protein, 85 aa, Ancylostoma caninum
KATMQCGENEKYDSCGSKECDKKCKYDGVEEEDDEEPNVPCLVRVCHQDCVCEEGFYRNKDDKCVSAEDCELDNMDFIYPGTRNP